European Patent Application EP 4 772 527 A1, published July 8, 2026. Title: Peptide Having Activity of Skin Whitening and Uses Thereof. Applicant: CAREGEN CO., LTD. The sequence listing filed with the application follows.

SEQUENCE LISTING (13 sequences)

SEQ ID NO: 1 - protein, 6 aa, synthetic construct
THTISR

SEQ ID NO: 2 - DNA, 21 bp, synthetic construct
  source 1..21: mol_type = other DNA
ccagcctggcgatcatgtcat

SEQ ID NO: 3 - DNA, 20 bp, synthetic construct
  source 1..20: mol_type = other DNA
ggtctggacaggagttgctg

SEQ ID NO: 4 - DNA, 20 bp, synthetic construct
  source 1..20: mol_type = other DNA
ggccagctttcaggcagagg

SEQ ID NO: 5 - DNA, 20 bp, synthetic construct
  source 1..20: mol_type = other DNA
tggtgcttcatgggcaaaat

SEQ ID NO: 6 - DNA, 20 bp, synthetic construct
  source 1..20: mol_type = other DNA
tctgtgaaggtgtgcaggag

SEQ ID NO: 7 - DNA, 20 bp, synthetic construct
  source 1..20: mol_type = other DNA
ccgaaacagagtggaaggtt

SEQ ID NO: 8 - DNA, 20 bp, synthetic construct
  source 1..20: mol_type = other DNA
ttctacattgtgggcgccat

SEQ ID NO: 9 - DNA, 20 bp, synthetic construct
  source 1..20: mol_type = other DNA
tcctccaggttggtcaatcg

SEQ ID NO: 10 - DNA, 20 bp, synthetic construct
  source 1..20: mol_type = other DNA
acgatgtcaggggcaaacat

SEQ ID NO: 11 - DNA, 20 bp, synthetic construct
  source 1..20: mol_type = other DNA
ctcctctgtgtcagcactgg

SEQ ID NO: 12 - DNA, 25 bp, synthetic construct
  source 1..25: mol_type = other DNA
ggtgtgaacggatttggccgtattg

SEQ ID NO: 13 - DNA, 25 bp, synthetic construct
  source 1..25: mol_type = other DNA
ccgttgaatttgccgtgagtggagt